European Patent Application EP 4 527 416 A1, published March 26, 2025. Title: 配体药物偶联物及其应用. Applicant: 成都百利多特生物药业有限责任公司. The sequence listing filed with the application follows.

SEQUENCE LISTING (10 sequences)

SEQ ID NO: 1 - protein, 219 aa, synthetic construct
DIQLTQSPSTLSASVGDRVTITCRASESLDNYGIRFLTWFQQKPGKAPKLLMYAASNQGSGVPSRFSGSGSGTEFTLTISSLQPDDFATYYCQQTKEVPWSFGQGTKVEVKRTVAAPSVFIFPPSDEQLKSGTASVVCLLNNFYPREAKVQWKVDNALQSGNSQESVTEQDSKDSTYSLSSTLTLSKADYEKHKVYACEVTHQGLSSPVCTKSFNRGEC

SEQ ID NO: 2 - protein, 445 aa, synthetic construct
EVQLVQSGAEVKKPGSSVKVSCKASGYTITDSNIHWVRQAPGQSLEWIGYIYPYNGGTDYNQKFKNRATLTVDNPTNTAYMELSSLRSEDTAFYYCVNGNPWLAYWGQGTLVTVSSASTKGPSVFPLAPSSKSTSGGTAALGCLVKDYFPEPVTVSWNSGALTSGVHTFPAVLQSSGLYSLSSVVTVPSSSLGTQTYICNVNHKPSNTKVDKRVEPKSCDKTHTCPPCPAPELLGGPSVFLFPPKPKDTLMISRTPEVTCVVVDVSHEDPEVKFNWYVDGVEVHNAKTKPREEQYNSTYRVVSVLTVLHQDWLNGKEYKCKVSNKALPAPIEKTISKAKGQPREPQVYTLPPSRDELTKNQVSLTCLVKGFYPSDIAVEWESNGQPENNYKTTPPVLDSDGSFFLYSKLTVDKSRWQQGNVFSCSVMHEALHNHYTQKSLSLSPG

SEQ ID NO: 3 - protein, 213 aa, synthetic construct
DIQMTQSPSSLSASVGDRVTITCRASQDINKYLAWYQQKPGKVPKLLIYSTSTLQSGVPSRFSGSGSGTDFTLTISSLQPEDVATYYCLQYDDLFTFGQGTKLEIKRTVAAPSVFIFPPSDEQLKSGTASVVCLLNNFYPREAKVQWKVDNALQSGNSQESVTEQDSKDSTYSLSSTLTLSKADYEKHKVYACEVTHQGLSSPVTKSFNRGEC

SEQ ID NO: 4 - protein, 447 aa, synthetic construct
QVQLVQSGAEVKKPGASVKLSCKASGYTFTSFDINWVRQAPEQRLEWMGWIFPGDGNTKYSQKFQGRATITRDTSASTAYMELSSLRSEDTAVYYCVRGEALYYFDYWGQGTLVTVSSASTKGPSVFPLAPSSKSTSGGTAALGCLVKDYFPEPVTVSWNSGALTSGVHTFPAVLQSSGLYSLSSVVTVPSSSLGTQTYICNVNHKPSNTKVDKRVEPKSCDKTHTCPPCPAPELLGGPSVFLFPPKPKDTLMISRTPEVTCVVVDVSHEDPEVKFNWYVDGVEVHNAKTKPREEQYNSTYRVVSVLTVLHQDWLNGKEYKCKVSNKALPAPIEKTISKAKGQPREPQVYTLPPSRDELTKNQVSLTCLVKGFYPSDIAVEWESNGQPENNYKTTPPVLDSDGSFFLYSKLTVDKSRWQQGNVFSCSVMHEALHNHYTQKSLSLSPG

SEQ ID NO: 5 - protein, 214 aa, synthetic construct
DIQMTQSPSSLSASVGDRVTITCRASQDINKYLAWYQQKPGKVPKLLIYSTSTLQSGVPSRFSGSGSGTDFTLTISSLQPEDVATYYCLQYDDLFTFGQGTKLEIKRTVAAPSVFIFPPSDEQLKSGTASVVCLLNNFYPREAKVQWKVDNALQSGNSQESVTEQDSKDSTYSLSSTLTLSKADYEKHKVYACEVTHQGLSSPVCTKSFNRGEC

SEQ ID NO: 6 - protein, 447 aa, synthetic construct; identical to SEQ ID NO: 4

SEQ ID NO: 7 - protein, 214 aa, synthetic construct
DIQMTQSPSSLSASVGDRVTITCRASQDVNTAVAWYQQKPGKAPKLLIYSASFLYSGVPSRFSGSRSGTDFTLTISSLQPEDFATYYCQQHYTTPPTFGQGTKVEIKRTVAAPSVFIFPPSDEQLKSGTASVVCLLNNFYPREAKVQWKVDNALQSGNSQESVTEQDSKDSTYSLSSTLTLSKADYEKHKVYACEVTHQGLSSPVTKSFNRGEC

SEQ ID NO: 8 - protein, 449 aa, synthetic construct
EVQLVESGGGLVQPGGSLRLSCAASGFNIKDTYIHWVRQAPGKGLEWVARIYPTNGYTRYADSVKGRFTISADTSKNTAYLQMNSLRAEDTAVYYCSRWGGDGFYAMDYWGQGTLVTVSSASTKGPSVFPLAPSSKSTSGGTAALGCLVKDYFPEPVTVSWNSGALTSGVHTFPAVLQSSGLYSLSSVVTVPSSSLGTQTYICNVNHKPSNTKVDKKVEPKSCDKTHTCPPCPAPELLGGPSVFLFPPKPKDTLMISRTPEVTCVVVDVSHEDPEVKFNWYVDGVEVHNAKTKPREEQYNSTYRVVSVLTVLHQDWLNGKEYKCKVSNKALPAPIEKTISKAKGQPREPQVYTLPPSREEMTKNQVSLTCLVKGFYPSDIAVEWESNGQPENNYKTTPPVLDSDGSFFLYSKLTVDKSRWQQGNVFSCSVMHEALHNHYTQKSLSLSPG

SEQ ID NO: 9 - protein, 215 aa, synthetic construct
DIQMTQSPSSLSASVGDRVTITCRASQDVNTAVAWYQQKPGKAPKLLIYSASFLYSGVPSRFSGSRSGTDFTLTISSLQPEDFATYYCQQHYTTPPTFGQGTKVEIKRTVAAPSVFIFPPSDEQLKSGTASVVCLLNNFYPREAKVQWKVDNALQSGNSQESVTEQDSKDSTYSLSSTLTLSKADYEKHKVYACEVTHQGLSSPVCTKSFNRGEC

SEQ ID NO: 10 - protein, 449 aa, synthetic construct; identical to SEQ ID NO: 8